European Patent Specification EP 3 612 630 B1, published August 30, 2023. Title: SITE-SPECIFIC DNA MODIFICATION USING A DONOR DNA REPAIR TEMPLATE HAVING TANDEM REPEAT SEQUENCES. Applicant: NELSON, JOHN RICHARD SMITH, ANJA SCHIEL, JOHN SPOONER, PATRICK MCCOY LOWERY, LISA DUTHIE, ROBERT. The sequence listing filed with the application follows.

SEQUENCE LISTING (11 sequences)

SEQ ID NO: 1 - DNA, 19 bp, Artificial Sequence
  Description of Artificial Sequence: Synthetic primer
actctgcttgaaagcttta

SEQ ID NO: 2 - DNA, 19 bp, Artificial Sequence
  Description of Artificial Sequence: Synthetic primer
taaagctttcaagcagagt

SEQ ID NO: 3 - DNA, 18 bp, Artificial Sequence
  Description of Artificial Sequence: Synthetic primer
ggtcctccgatcgttgtc

SEQ ID NO: 4 - DNA, 18 bp, Artificial Sequence
  Description of Artificial Sequence: Synthetic primer
gacaacgatcggaggacc

SEQ ID NO: 5 - DNA, 21 bp, Artificial Sequence
  Description of Artificial Sequence: Synthetic primer
ctaagagctttggtatccccc

SEQ ID NO: 6 - DNA, 20 bp, Artificial Sequence
  Description of Artificial Sequence: Synthetic primer
ctgcaactttaaatgggccc

SEQ ID NO: 7 - DNA, 6 bp, Artificial Sequence
  Description of Artificial Sequence: Synthetic primer
  modified_base (1)..(6): a, c, t, g, unknown or other
nnnnnn

SEQ ID NO: 8 - DNA, 56 bp, Artificial Sequence
  Description of Artificial Sequence: Synthetic primer
gcgcgcgctagccgatcggattacacgatcattcgactgcaactttaaatgggccc

SEQ ID NO: 9 - DNA, 33 bp, Artificial Sequence
  Description of Artificial Sequence: Synthetic primer
gcgcgcactagtctaagagctttggtatccccc

SEQ ID NO: 10 - DNA, 52 bp, Artificial Sequence
  Description of Artificial Sequence: Synthetic primer
gcgcgcgctagccgatcggattacacgatcattcgaagtgctgagcaggcag

SEQ ID NO: 11 - DNA, 34 bp, Artificial Sequence
  Description of Artificial Sequence: Synthetic primer
gcgcgcactagtcccaccattccttatatcctcc